European Patent Application EP 4 353 821 A1, published April 17, 2024. Title: Transposase mutant with enhanced efficienc of gene transfer. Applicant: Max-Delbrueck-Centrum fuer Molekulare Medizin in der Helmholtz-Gemeinschaft. Application EP. The sequence listing filed with the application follows.

SEQUENCE LISTING (27 sequences)

SEQ ID NO: 1 - protein, 340 aa, synthetic construct
  source 1..340: note = SB 100X
MGKSKEISQDLRKKIVDLHKSGSSLGAISKRLKVPRSSVQTIVRKYKHHGTTQPSYRSGRRRVLSPRDERTLVRKVQINPRTTAKDLVKMLEETGTKVSISTVKRVLYRHNLKGRSARKKPLLQNRHKKARLRFATAHGDKDRTFWRNVLWSDETKIELFGHNDHRYVWRKKGEACKPKNTIPTVKHGGGSIMLWGCFAAGGTGALHKIDGIMRKENYVDILKQHLKTSVRKLKLGRKWVFQMDNDPKHTSKVVAKWLKDNKVKVLEWPSQSPDLNPIENLWAELKKRVRARRPTNLTQLHQLCQEEWAKIHPTYCGKLVEGYPKRLTQVKQFKGNATKY

SEQ ID NO: 2 - protein, 339 aa, synthetic construct
  source 1..339: note = Tdr1
MGKSKEISQDIRKRIVDLHKSGSSLVTISRCLKVPHSSVQTNLRNYKQHGNVQPSYRSGRRRILCPRDERAMVRTVCINPRTKAKDLVKMLAEAGKRVSLSTVKRVLYHGLKGHSARKKPLLQKHHKKARLQFAKLHWEKDLCFWRHVLWSDGAKIELFGHNDQRYIWRTKGKAYKPKNTIPTVQYGGGSIMLWGCFAAGGTGPLHSIDGIMRKEHYVEILKQHLKTSARKLKLGHKWVFQMDHDPKHTAKLVKMCFKDNRVNVLEWPSQSPDLNPIENLWAELKKLVRARQPTNLTQLHQFCQEEWAKIPANYCEKLVEGYPKHLTKVIQFKSKAYKY

SEQ ID NO: 3 - protein, 340 aa, synthetic construct
  source 1..340: note = ZB
MGKNKELSQDLRSLIVEKHFDGNGYRRISRMLNVPVSTVGAIIRKWKKHKFTINRPRSGAPRKIPVRGVQRIIRRVLQEPRTTRAELQEDLASAGTIVSKKTISNALNHHGIHARSPRKTPLLNKKHVEARLKFAKQHLEKPVDYWETIVWSDESKIELFGSHSTHHVWRRNGTAHHPKNTIPTVKFGGGSIMVWGCFSARGTGRLHIIEGRMNGEMYRDILDKNLLPSTRKLKMKRGWTFQQDNDPKHKAKETMKWFQRKKIKLLEWPSQSPDLNPIENLWRELKIKVHKRGPRNLQDLKTVCVEEWARITPEQCRRLVSPYKRRLEAVITNKGFSTKY

SEQ ID NO: 4 - protein, 340 aa, synthetic construct
  source 1..340: note = FP
MPRPKEIQEQLRKKVIEIYQSGKGYKAISKALGIQRTTVRAIIHKWRRHGTVVNLPRSGRPPKITPRAQRRLIQEVTKDPTTTSKELQASLASVKVSVHASTIRKRLGKNGLHGRVPRRKPLLSKKNIKARLNFSTTHLDDPQDFWDNILWTDETKVELFGRCVSKYIWRRRNTAFHKKNIIPTVKYGGGSVMVWGCFAASGPGRLAVIKGTMNSAVYQEILKENVRPSVRVLKLKRTWVLQQDNDPKHTSKSTTEWLKKNKMKTLEWPSQSPDLNPIEMLWYDLKKAVHARKPSNVTELGQFCKDEWAKIPPGRCKSLIARYRKRLVAVVAAKGGPTSY

SEQ ID NO: 5 - protein, 339 aa, synthetic construct
  source 1..339: note = Passport
MKTKELTKQVRDKVVEKYEAGLGYKKISRALNISLSTIKSIIRKWKEYGTTANLPRGGRPPKLKSRTRRKLIREATRRPMVTLEELQRSTAEVGESVHRTTISRLLHKSGLYGRVARRKPLLKGIHKKSRLEFARSHVGDTANMWKKVLWSDETKIELFGLNAKRYVWRKPNTAHHPEHTIPTVKHGGGSIMLWGCFSSAGTGKLVRIEGKMDGAKYREILEENLMQSAKDLRLGRRFIFQQDNDPKHTARATKEWFGLKNVNVLKWPSQSPDLNPIENLWQDLKIAVHRRSPSNLTELHLFCQEEWTNLSISRCAKLVETYPKRLAAVIAAKGGSTKY

SEQ ID NO: 6 - protein, 340 aa, synthetic construct
  source 1..340: note = TCB2
MARLSTATRHKVVILHQQGLSQAEISRQTGVSRCAVQALLKKHKETGNVEDRRRSGRPRKLTAADERHIMLTSLCNRKMSSSAISSELAENSGTEGHPSTVRRSLVRSGLHGRLAAKKPYLRRGNKAKRLNYARKHRNWGAKWQQVLWTDESKFEIFGCSRRQFVRRRAGERYTNECLQATVKHGGGSLQVWGCISANGVGDLVRINGLLNAEKYRQILIHHAIPSGRHLIGPKFILQHDNDPKHTAKVIKNYLQRKEEQGVLEVMVWPPQSPDLNIIESVWDYMKREKQLRLPKSTEELWLVLQDVWANLPAEFLQKLCASVPRRIDAVLKAKGGHTKY

SEQ ID NO: 7 - protein, 345 aa, synthetic construct
  source 1..345: note = S
MPGKRLAFEVTQLIYYNHQLGKSIPELVEIFSVSRKTVYNILNRAEKEGRLEPKSGGGCKTKINKRVDRLIMRKAIANPRISVRSLAQDIREECHLTVSHETVRQVILRHRYSSRVARKKPLLSEINIEKRHSFAVSMMDHAEEYWDDVIFCDETKMMLFYNDGPSRVWRKPLSALETQNIIPTIKFGKLSVMIWGCISSHGVGKLAFIESTMNAVQYLDILKTNLKASAEKFGLFSNNKPNFKFYQDNDPKHKEYNVRNWLLYNCGKVIDTPPQSPDLNPIENLWAYLKKKVAKRGPKTRQQLMAAIIAAWEKIPLEYDLKKLIHSMKKRLQLVAKANGGHTKY

SEQ ID NO: 8 - protein, 342 aa, synthetic construct
  source 1..342: note = Quetzal
MTREELSVSKRQDIIRLHGAQGKSYTEIAMLTNINRNTVARVIQRYKYEGRVSNLPRKGRPSVCTDRMRRAIKRLVDAEPEISAQSVAIVLNERHGIAISCETVRRYIHKFGYKAYNRRKKPQISPINRKRRLEFAKKYVNHPPEFWKKVLFTDESKFNIFGWDGTIKVWRPPGEGLNPKYTAKTVKHNGGGVLVWGCMAANGVGNLQVIDGIMDQYVYINILKQNLGPSLEKLGMSQDYWFQQDNDPKHTAFNSRLFLLYNTPHQLKSPPQSPDLNPIEHAWELLERKIWQTRIKNRVDLENKLKEAWITISEDYTQNLVNSMPERRLAEVIKMKGYATRY

SEQ ID NO: 9 - protein, 348 aa, synthetic construct
  source 1..348: note = Paris
MPGQRINENVIQLVYFHYHKGKCAKELAEMFSIKLRTIYNIINRAEKENRLELKHSGGRPAKLSRRDHSKILKQINENPQTSLRQLALDLKNDCNKTVSHETVRKVLKMHKYSSQIARKKPLLSAVNIQRRLNFSITNVNKPAEYWDDVIFCDETKIMLYYHDGPSKVWRKPNTALEQKNIIPTVKFGKLSVMVWGCISSKGVGELRIFNDVMTKEFYLDILKNELSRSAIKFGFVDPQNPSKQRYKLYQDNDPKHKSFLCRTWLLYNCSKVIDTPAQSPDLNPIENLWAFLKKRVGKRSPTNKNALIKAIQEEWIKIPEIYDLHNLIQSMSRRLRAVMDANGQYTKY

SEQ ID NO: 10 - protein, 343 aa, synthetic construct
  source 1..343: note = Tc1
MVKSVGCKNLSLDVKKAIVAGFEQGIPTKMLALQIQRSPSTIWKVIKKYQTEKSVALRISPGRPRVTTHRMDRNILRSAREDPHRTATDIQMIISSPNEPVPSKRTVRRRLQQAGLHGRKPVKKPFISKKNRMARVAWAKAHLRWGRQEWAKHIWSDESKFNLFGSDGNSWVRRPVGSRYSPKYQCPTVKHGGGSVMVWGCFTSTSMGPLRRIQSIMDRFQYENIFETTMRPWALQNVGRGFVFQQDNDPKHTSLHVRSWFQRRHVHLLDWPSQSPDLNPIEHLWEELERRLGGIRASNADAKFNQLENAWKAIPMSVIHKLIDSMPRRCQAVIDANGYATKY

SEQ ID NO: 11 - protein, 341 aa, synthetic construct
  source 1..341: note = Minos
MVRGKPISKEIRVLIRDYFKSGKTLTEISKQLNLPKSSVHGVIQIFKKNGNIENNIANRGRTSAITPRDKRQLAKIVKADRRQSLRNLASKWSQTIGKTVKREWTRQQLKSIGYGFYKAKEKPLLTLRQKKKRLQWARERMSWTQRQWDTIIFSDEAKFDVSVGDTRKRVIRKRSETYHKDCLKRTTKFPASTMVWGCMSAKGLGKHLFIEGTVNAEKYINILQDSLLPSIPKLLDCGEFTFQQDGASSHTAKRTKNWLQYNQMEVLDWPSNSPDLSPIENIWWLMKNQLRNEPQRNISDLKIKLQEMWDSISQEHCKNLLSSMPKRVKCVMQAKGDVTQF

SEQ ID NO: 12 - protein, 337 aa, synthetic construct
  source 1..337: note = Uhu
MGKRTTIEQRKLILEHFKIGYSYRQIAKMVNLSTTTVFNIIRRFVDENRIEDKGRKAPNKIFTEQEERRRIIRKIRENPKLSAPKLTQQVQDEMGKKCSVQTVRRVLHNHDFNARVPRKKPFISTKNKGTRMTFAKTHLDKDLEFWNTIIFEDESKFIIFGSDGRNYVRRQSNTELNPKNLKATVKHGGSVMVWACISAASVGNLVCIETTTDRNVDLSILKENLLQSAEKLGIRRYFRFYQDNDQTTTKHKSGLVPSWLIWNCPHMIIPAQSPDVNVINLWDLLENNIIRNHRSNLKNALLDEWSKISPETTRKLVSSMNNRLMEDIKAKGYHTKY

SEQ ID NO: 13 - protein, 339 aa, synthetic construct
  source 1..339: note = Bari
MPKTKELTVEARAGIVARFKAGTPAAKIAEIYQISRRTVYYLIKKFDTVGTLKNKKRSGRKPVLDQRQCRQILGVVAKNPSASPVKIALESKNTIGKQVSSSTIRRRLKEADFKTYVVRKTIEITPTNKTKRLRFALEYVKKPLDFWFNILWTDESAFQYQGSYSKHFMHLKNNQKHLAAQPTNRFGGGTVMFWGCLSYYGFGDLVPIEGTLNQNGYLLILNNHAFTSGNRLFPTTEWILQQDNAPCHKGRIPTKFLNDLNLAVLPWPPQSPDLNIIENVWAFIKNQRTIDKNRKREGAIIEIAEIWSKLTLEFAQTLVRSIPKRLQAVIDAKGGVTKY

SEQ ID NO: 14 - protein, 326 aa, synthetic construct
  source 1..326: note = Tc3
MPRGSALSDTERAQDVMKLLNVSLHEMSRKISRSRHCIREYLKDPVSYGTSKRAPRRKALSVRDERNVIRAASNSCKTARDIRNELQLSASKRTILNVIKRSGVIVRQKLRPAPLLSADHKLKRLEFAKNMTNWSKVVFSDEKKFNLDGPDGCRYYWRDLRKEPMVFSRRNFGGGTVMVWGAFTEKKKLEIQFVSSKMNSTDYQNVLELELSKYLRHYSRKDFRFQQDNATIHVSNSTRDYFKLKKINLLDWPARSPDLNPIENLWGILVRIVYAQNKTYPTVASLKQGILDAWKSIPDNQLKSLVRSMEDRLIEIIRTQGNPINY

SEQ ID NO: 15 - protein, 311 aa, synthetic construct
  source 1..311: note = Impala
MPRGKELTPSLRSRICELKKQGYSYSQIHKHFPYIPLGTIKTTCRRAQRGAENTTLPRSGAPRKPHEEQRDQIYDTVITDPHVTTRDLLDSVDNVIKKRSLRYLLREMNKRKWIQKKRVALTPLQARKRLDWAIRYQGIDWRRVKWSDECMVRRGQGMRPIWTFLSPREPYAYRMFKKLGGRSCRQMFWAAFGHRSRTPLVPLVGKLNAIGIYELYSFILPWFLQSGDIFMHDNASVHTARIVKALLEELGVDLMTWPPYSPDLNPIENLWALMKAEIYRLHPELTHTEDTVATQHALVLAAMEAWDNIED

SEQ ID NO: 16 - protein, 348 aa, synthetic construct
  source 1..348: note = Himar
MEKKEFRVLIKYCFLKGKNTVEAKTWLDNEFPDSAPGKSTIIDWYAKFKRGEMSTEDGERSGRPKEVVTDENIKKIHKMILNDRKMKLIEIAEALKISKERVGHIIHQYLDMRKLCAKWVPRELTFDQKQQRVDDSERCLQLLTRNTPEFFRRYVTMDETWLHHYTPESNRQSAEWTATGEPSPKRGKTQKSAGKVMASVFFDAHGIIFIDYLEKGKTINSDYYMALLERLKVEIAAKRPHMKKKKVLFHQDNAPCHKSLRTMAKIHELGFELLPHPPYSPDLAPSDFFLFSDLKRMLAGKKFGCNEEVIAETEAYFEAKPKEYYQNGIKKLEGRYNRCIALEGNYVE

SEQ ID NO: 17 - protein, 345 aa, synthetic construct
  source 1..345: note = Mos1
MSSFVPNKEQTRTVLIFCFHLKKTAAESHRMLVEAFGEQVPTVKTCERWFQRFKSGDFDVDDKEHGKPPKRYEDAELQALLDEDDAQTQKQLAEQLEVSQQAVSNRLREMGKIQKVGRWVPHELNERQMERRKNTCEILLSRYKRKSFLHRIVTGDEKWIFFVNPKRKKSYVDPGQPATSTARPNRFGKKTMLCVWWDQSGVIYYELLKPGETVNTARYQQQLINLNRALQRKRPEYQKRQHRVIFLHDNAPSHTARAVRDTLETLNWEVLPHAAYSPDLAPSDYHLFASMGHALAEQRFDSYESVKKWLDEWFAAKDDEFYWRGIHKLPERWEKCVASDGKYFE

SEQ ID NO: 18 - protein, 340 aa, synthetic construct
  source 1..340: note = SB100X Q124X not Q
  VARIANT 124: note = X is not Q
MGKSKEISQDLRKKIVDLHKSGSSLGAISKRLKVPRSSVQTIVRKYKHHGTTQPSYRSGRRRVLSPRDERTLVRKVQINPRTTAKDLVKMLEETGTKVSISTVKRVLYRHNLKGRSARKKPLLXNRHKKARLRFATAHGDKDRTFWRNVLWSDETKIELFGHNDHRYVWRKKGEACKPKNTIPTVKHGGGSIMLWGCFAAGGTGALHKIDGIMRKENYVDILKQHLKTSVRKLKLGRKWVFQMDNDPKHTSKVVAKWLKDNKVKVLEWPSQSPDLNPIENLWAELKKRVRARRPTNLTQLHQLCQEEWAKIHPTYCGKLVEGYPKRLTQVKQFKGNATKY

SEQ ID NO: 19 - protein, 340 aa, synthetic construct
  source 1..340: note = SB100X Q124C
MGKSKEISQDLRKKIVDLHKSGSSLGAISKRLKVPRSSVQTIVRKYKHHGTTQPSYRSGRRRVLSPRDERTLVRKVQINPRTTAKDLVKMLEETGTKVSISTVKRVLYRHNLKGRSARKKPLLCNRHKKARLRFATAHGDKDRTFWRNVLWSDETKIELFGHNDHRYVWRKKGEACKPKNTIPTVKHGGGSIMLWGCFAAGGTGALHKIDGIMRKENYVDILKQHLKTSVRKLKLGRKWVFQMDNDPKHTSKVVAKWLKDNKVKVLEWPSQSPDLNPIENLWAELKKRVRARRPTNLTQLHQLCQEEWAKIHPTYCGKLVEGYPKRLTQVKQFKGNATKY

SEQ ID NO: 20 - protein, 340 aa, synthetic construct
  REGION 1..340: note = SB100X Q124C H187V
MGKSKEISQDLRKRIVDLHKSGSSLGAISKRLAVPRSSVQTIVRKYKHHGTTQPSYRSGRRRVLSPRDERTLVRKVQINPRTTAKDLVKMLEETGTKVSISTVKRVLYRHNLKGHSARKKPLLCNRHKKARLRFATAHGDKDRTFWRNVLWSDETKIELFGHNDHRYVWRKKGEACKPKNTIPTVKVGGGSIMLWGCFAAGGTGALHKIDGIMDAVQYVDILKQHLKTSVRKLKLGRKWVFQHDNDPKHTSKVVAKWLKDNKVKVLEWPSQSPDLNPIENLWAELKKRVRARRPTNLTQLHQLCQEEWAKIHPNYCGKLVEGYPKRLTQVKQFKGNATKY

SEQ ID NO: 21 - protein, 340 aa, synthetic construct
  REGION 1..340: note = SB100X Q124C P247R
MGKSKEISQDLRKRIVDLHKSGSSLGAISKRLAVPRSSVQTIVRKYKHHGTTQPSYRSGRRRVLSPRDERTLVRKVQINPRTTAKDLVKMLEETGTKVSISTVKRVLYRHNLKGHSARKKPLLCNRHKKARLRFATAHGDKDRTFWRNVLWSDETKIELFGHNDHRYVWRKKGEACKPKNTIPTVKHGGGSIMLWGCFAAGGTGALHKIDGIMDAVQYVDILKQHLKTSVRKLKLGRKWVFQHDNDRKHTSKVVAKWLKDNKVKVLEWPSQSPDLNPIENLWAELKKRVRARRPTNLTQLHQLCQEEWAKIHPNYCGKLVEGYPKRLTQVKQFKGNATKY

SEQ ID NO: 22 - protein, 340 aa, synthetic construct
  REGION 1..340: note = transposase with substitution K248R
MGKSKEISQDLRKRIVDLHKSGSSLGAISKRLAVPRSSVQTIVRKYKHHGTTQPSYRSGRRRVLSPRDERTLVRKVQINPRTTAKDLVKMLEETGTKVSISTVKRVLYRHNLKGHSARKKPLLQNRHKKARLRFATAHGDKDRTFWRNVLWSDETKIELFGHNDHRYVWRKKGEACKPKNTIPTVKHGGGSIMLWGCFAAGGTGALHKIDGIMDAVQYVDILKQHLKTSVRKLKLGRKWVFQHDNDPRHTSKVVAKWLKDNKVKVLEWPSQSPDLNPIENLWAELKKRVRARRPTNLTQLHQLCQEEWAKIHPNYCGKLVEGYPKRLTQVKQFKGNATKY

SEQ ID NO: 23 - DNA, 19 bp, synthetic construct
  source 1..19: mol_type = other DNA; note = SB100X-Q124_to_C-rev
cttcttccttgctgagtgg

SEQ ID NO: 24 - DNA, 30 bp, synthetic construct
  source 1..30: mol_type = other DNA; note = SB100X-Q124_to_C124-fwd
ccactgctctgcaaccgacataagaaagcc

SEQ ID NO: 25 - protein, 6 aa, synthetic construct
  source 1..6: note = WVPHEL motif
WVPHEL

SEQ ID NO: 26 - protein, 5 aa, synthetic construct
  source 1..5: note = KKPLL
KKPLL

SEQ ID NO: 27 - protein, 7 aa, synthetic construct
  source 1..7: note = ARKKPLL motif
ARKKPLL